European Patent Application EP 4 144 856 A1, published March 8, 2023. Title: Retroviral Vector Producer Cell and Packaging Cell and Preparation Method Thereof. Applicant: Shenzhen Eureka Biotechnology Co., LTD. The sequence listing filed with the application follows.

SEQUENCE LISTING (59 sequences)

SEQ ID NO: 1 - DNA, 1893 bp, Artificial sequence
  18BF003_pma-MCS
actgcggccgccctgcaggtcaactagtgacgtcttaattaattgccggctggaacgcgtttcgaacatcgattgaattctggccaagtggatccgctagctctagagtcgacggtaccaagcttgcctcgagccatggagatctgcatgccctaggtccggaaccggttggcgcgccatctggcagcgatcgccgcggaacccctatttgtttatttttctaaatacattcaaatatgtatccgctcatgagacaataaccctgataaatgcttcaataatattgaaaaaggaagagtatgagtattcaacatttccgtgtcgcccttattcccttttttgcggcattttgccttcctgtttttgctcacccagaaacgctggtgaaagtaaaagatgctgaagatcagttgggtgcacgagtgggttacatcgaactggatctcaacagcggtaagatccttgagagttttcgccccgaagaacgttttccaatgatgagcacttttaaagttctgctatgtggcgcggtattatcccgtattgacgccgggcaagagcaactcggtcgccgcatacactattctcagaatgacttggttgagtactcaccagtcacagaaaagcatcttacggatggcatgacagtaagagaattatgcagtgctgccataaccatgagtgataacactgcggccaacttacttctgacaacgatcggaggaccgaaggagctaaccgcttttttgcacaacatgggggatcatgtaactcgccttgatcgttgggaaccggagctgaatgaagccataccaaacgacgagcgtgacaccacgatgcctgtagcaatggcaacaacgttgcgcaaactattaactggcgaactacttactctagcttcccggcaacaattaatagactggatggaggcggataaagttgcaggaccacttctgcgctcggcccttccggctggctggtttattgctgataaatctggagccggtgagcgtgggtctcgcggtatcattgcagcactggggccagatggtaagccctcccgtatcgtagttatctacacgacggggagtcaggcaactatggatgaacgaaatagacagatcgctgagataggtgcctcactgattaagcattggtaacgtacggaagttagagaaaaggcataagtagaaaagatcaaaggatcttcttgagatcctttttttctgcgcgtaatctgctgcttgcaaacaaaaaaaccaccgctaccagcggtggtttgtttgccggatcaagagctaccaactctttttccgaaggtaactggcttcagcagagcgcagataccaaatactgttcttctagtgtagccgtagttaggccaccacttcaagaactctgtagcaccgcctacatacctcgctctgctaatcctgttaccagtggctgctgccagtggcgataagtcgtgtcttaccgggttggactcaagacgatagttaccggataaggcgcagcggtcgggctgaacggggggttcgtgcacacagcccagcttggagcgaacgacctacaccgaactgagatacctacagcgtgagctatgagaaagcgccacgcttcccgaagggagaaaggcggacaggtatccggtaagcggcagggtcggaacaggagagcgcacgagggagcttccagggggaaacgcctggtatctttatagtcctgtcgggtttcgccacctctgacttgagcgtcgatttttgtgatgctcgtcaggggggcggagcctatggaaaaacgccagcaacgcggcctttttacggttcctggccttttgctggccttttgctcatctcatgaaaattatgcaaattgagccagtcaggcagt

SEQ ID NO: 2 - DNA, 2900 bp, Artificial sequence
  NotI-IR/DR-HS4I-CMV-BGI-MCS-hGHpA-HS4I-IR/DR-AsiSI
gcggccgcatctatacagttgaagtcggaagtttacatacacttaagttggagtcattaaaactcgtttttcaactactccacaaatttcttgttaacaaacaatagttttggcaagtcagttaggacatctactttgtgcatgacacaagtcatttttccaacaattgtttacagacagattatttcacttataattcactgtatcacaattccagtgggtcagaagtttacatacactaagttgactgtgcctttaaacagcttggaaaattccagaaaatgatgtcatggctttagcctgcagggagggacagcccccccccaaagcccccagggatgtaattacgtccctcccccgctagggggcagcagcgagccgcccggggctccgctccggtccggcgctccccccgcatccccgagccggcagcgtgcggggacagcccgggcacggggaaggtggcacgggatcgctttcctctgaacgcttctcgctgctctttgagcctgcagacacctggggggatacggggaaaaggacctgcaggtcaactagtgacgtcttaattaattgccggctggacgtacgcgtctagttattaatagtaatcaattacggggtcattagttcatagcccatatatggagttccgcgttacataacttacggtaaatggcccgcctggctgaccgcccaacgacccccgcccattgacgtcaataatgacgtatgttcccatagtaacgccaatagggactttccattgacgtcaatgggtggagtatttacggtaaactgcccacttggcagtacatcaagtgtatcatatgccaagtacgccccctattgacgtcaatgacggtaaatggcccgcctggcattatgcccagtacatgaccttatgggactttcctacttggcagtacatctacgtattagtcatcgctattaccatggtgatgcggttttggcagtacatcaatgggcgtggatagcggtttgactcacggggatttccaagtctccaccccattgacgtcaatgggagtttgttttggcaccaaaatcaacgggactttccaaaatgtcgtaacaactccgccccattgacgcaaatgggcggtaggcgtgtacggtgggaggtctatataagcagagctcgtttagtgaaccgtcagatcgcctggagacgccatccacgctgttttgacctccatagaagacaccgggaccgatccagcctccgcggattcgaatcccggccgggaacggtgcattggaacgcggattccccgtgccaagagtgacgtaagtaccgcctatagagtctataggcccacaaaaaatgctttcttcttttaatatacttttttgtttatcttatttctaatactttccctaatctctttctttcagggcaataatgatacaatgtatcatgcctctttgcaccattctaaagaataacagtgataatttctgggttaaggcaatagcaatatttctgcatataaatatttctgcatataaattgtaactgatgtaagaggtttcatattgctaatagcagctacaatccagctaccattctgcttttattttatggttgggataaggctggattattctgagtccaagctaggcccttttgctaatcatgttcatacctcttatcttcctcccacagctcctgggcaacgtgctggtctgtgtgctggcccatcactttggcaaagaattgggattcgaacatcgattgaattctggccaggatccgctagctctagagtcgacggtaccagtactaagcttgcctcgagccatggagatctacgggtggcatccctgtgacccctccccagtgcctctcctggccctggaagttgccactccagtgcccaccagccttgtcctaataaaattaagttgcatcattttgtctgactaggtgtccttctataatattatggggtggaggggggtggtatggagcaaggggcaagttgggaagacaacctgtagggcctgcggggtctattgggaaccaagctggagtgcagtggcacaatcttggctcactgcaatctccgcctcctgggttcaagcgattctcctgcctcagcctcccgagttgttgggattccaggcaagcatgaccaggctcagctaatttttgtttttttggtagagacggggtttcaccatattggccaggctggtctccaactcctaatctcaggtgatctacccaccttggcctcccaaattgctgggattacaggcgtgaaccactgctcccttccctgtccttgcatgccctaggcagctgtccggaaccggtgtttaaacaggccttttccccgtatccccccaggtgtctgcaggctcaaagagcagcgagaagcgttcagaggaaagcgatcccgtgccaccttccccgtgcccgggctgtccccgcacgctgccggctcggggatgcggggggagcgccggaccggagcggagccccgggcggctcgctgctgccccctagcgggggagggacgtaattacatccctgggggctttgggggggggctgtccctcaggccttggcgcgccctaaagccatgacatcattttctggaattttccaagctgtttaaaggcacagtcaacttagtgtatgtaaacttctgacccactggaattgtgatacagtgaattataagtgaaataatctgtctgtaaacaattgttggaaaaatgacttgtgtcatgcacaaagtagatgtcctaactgacttgccaaaactattgtttgttaacaagaaatttgtggagtagttgaaaaacgagttttaatgactccaacttaagtgtatgtaaacttccgacttcaactgtatagcgatcgc

SEQ ID NO: 3 - DNA, 1386 bp, Artificial sequence
  NotI-PB3'ITR-HS4I-MCS-HS4I-PB5'ITR-AsiSI
gcggccgcaacacgcagctagattaaccctagaaagataatcatattgtgacgtacgttaaagataatcatgcgtaaaattgacgcatgtgttttatcggtctgtatatcgaggtttatttattaatttgaatagatattaagttttattatatttacacttacatactaataataaattcaacaaacaatttatttatgtttatttatttattaaaaaaaaacaaaaactcaaaatttcttctataaagtaacaaaacttttatcctgcagggagggacagcccccccccaaagcccccagggatgtaattacgtccctcccccgctagggggcagcagcgagccgcccggggctccgctccggtccggcgctccccccgcatccccgagccggcagcgtgcggggacagcccgggcacggggaaggtggcacgggatcgctttcctctgaacgcttctcgctgctctttgagcctgcagacacctggggggatacggggaaaaggacctgcaggtcaactagtgacgtcttaattaattgccggctggacgtacgcgttttggcaaaatcgattgaattctggccaagtggatccgctagctctagagtcgacggtaccagtactaagcttgcctcgaggatatcccatggagatctatggggacatcatgaagccccttgagcatctgacttctggctaataaaggaaatttattttcattgcaatagtgtgttggaattttttgtgtctctcactcggaaggacatatgggagcatgccctaggcagctgtccggaaccggtgtttaaacaggccttttccccgtatccccccaggtgtctgcaggctcaaagagcagcgagaagcgttcagaggaaagcgatcccgtgccaccttccccgtgcccgggctgtccccgcacgctgccggctcggggatgcggggggagcgccggaccggagcggagccccgggcggctcgctgctgccccctagcgggggagggacgtaattacatccctgggggctttgggggggggctgtccctcaggccttggcgcgccatatctataacaagaaaatatatatataataagttatcacgtaagtagaacacgaaataacaatataattatcgtatgagttaaatcttaaaagtcacgtaaaagataatcatgcgtcattttgactcacgcggttgttatagttcaaaatcagtgacacttaccgcattgacaagcacgcctcacgggagctccaagcggcgactgagatgtcctaaatgcacagcgacggattcgcgctatttagaaagagagagcaatatttcaagaatgcatgcgtcaattttacgcagactatctttctagggttaagcgatcgc

SEQ ID NO: 4 - DNA, 915 bp, Artificial sequence
  MluI-TRE3GCuO-BGI-ClaI-EcoRI
acgcgttactccctatcagtgatagagaacgtatgaagagtttactccctatcagtgatagagaacgtatgcagactttactccctatcagtgatagagaacgtataaggagtttactccctatcagtgatagagaacgtatgaccagtttactccctatcagtgatagagaacgtatctacagtttactccctatcagtgatagagaacgtatatccagtttactccctatcagtgatagagaacgtattaggcgtgtacggtgggcgcctataaaagcagagctcgtttagtgaaccgtcagatcgcctggagcaattccacatacaaacagaccagattgtctgtttgttacacttttgtcttataccaactttccgtaccacttcctaccctcgtaaattcgaatcccggccgggaacggtgcattggaacgcggattccccgtgccaagagtgacgtaagtaccgcctatagagtctataggcccacaaaaaatgctttcttcttttaatatacttttttgtttatcttatttctaatactttccctaatctctttctttcagggcaataatgatacaatgtatcatgcctctttgcaccattctaaagaataacagtgataatttctgggttaaggcaatagcaatatttctgcatataaatatttctgcatataaattgtaactgatgtaagaggtttcatattgctaatagcagctacaatccagctaccattctgcttttattttatggttgggataaggctggattattctgagtccaagctaggcccttttgctaatcatgttcatacctcttatcttcctcccacagctcctgggcaacgtgctggtctgtgtgctggcccatcactttggcaaagaattgggattcgaaatcgattgaattc

SEQ ID NO: 5 - DNA, 887 bp, Artificial sequence
  MluI-TRE3G-BGI-ClaI-EcoRI
acgcgttactccctatcagtgatagagaacgtatgaagagtttactccctatcagtgatagagaacgtatgcagactttactccctatcagtgatagagaacgtataaggagtttactccctatcagtgatagagaacgtatgaccagtttactccctatcagtgatagagaacgtatctacagtttactccctatcagtgatagagaacgtatatccagtttactccctatcagtgatagagaacgtattaggcgtgtacggtgggcgcctataaaagcagagctcgtttagtgaaccgtcagatcgcctggagcaattccacaacacttttgtcttataccaactttccgtaccacttcctaccctcgtaaattcgaatcccggccgggaacggtgcattggaacgcggattccccgtgccaagagtgacgtaagtaccgcctatagagtctataggcccacaaaaaatgctttcttcttttaatatacttttttgtttatcttatttctaatactttccctaatctctttctttcagggcaataatgatacaatgtatcatgcctctttgcaccattctaaagaataacagtgataatttctgggttaaggcaatagcaatatttctgcatataaatatttctgcatataaattgtaactgatgtaagaggtttcatattgctaatagcagctacaatccagctaccattctgcttttattttatggttgggataaggctggattattctgagtccaagctaggcccttttgctaatcatgttcatacctcttatcttcctcccacagctcctgggcaacgtgctggtctgtgtgctggcccatcactttggcaaagaattgggattcgaaatcgattgaattc

SEQ ID NO: 6 - DNA, 897 bp, Artificial sequence
  MluI-TREadvCuO-BGI-ClaI-EcoRI
acgcgtgacgaggatcgttcgagcgagtttactccctatcagtgatagagaacgtatgtcgagtttactccctatcagtgatagagaacgatgtcgagtttactccctatcagtgatagagaacgtatgtcgagtttactccctatcagtgatagagaacgtatgtcgagtttactccctatcagtgatagagaacgtatgtcgagtttatccctatcagtgatagagaacgtatgtcgagtttactccctatcagtgatagagaacgtatgtcgaggtaggcgtgtacggtgggaggcctatataagcaaccggtgtttagtgaaccgtcagatcgcctggagacgccatcataatacaaacagaccagattgtctgtttgttttcgaatcccggccgggaacggtgcattggaacgcggattccccgtgccaagagtgacgtaagtaccgcctatagagtctataggcccacaaaaaatgctttcttcttttaatatacttttttgtttatcttatttctaatactttccctaatctctttctttcagggcaataatgatacaatgtatcatgcctctttgcaccattctaaagaataacagtgataatttctgggttaaggcaatagcaatatttctgcatataaatatttctgcatataaattgtaactgatgtaagaggtttcatattgctaatagcagctacaatccagctaccattctgcttttattttatggttgggataaggctggattattctgagtccaagctaggcccttttgctaatcatgttcatacctcttatcttcctcccacagctcctgggcaacgtgctggtctgtgtgctggcccatcactttggcaaagaattgggattcgaaatcgattgaattc

SEQ ID NO: 7 - DNA, 852 bp, Artificial sequence
  MluI-TREadv-BGI-ClaI-EcoRI
acgcgtgacgaggatcgttcgagcgagtttactccctatcagtgatagagaacgtatgtcgagtttactccctatcagtgatagagaacgatgtcgagtttactccctatcagtgatagagaacgtatgtcgagtttactccctatcagtgatagagaacgtatgtcgagtttactccctatcagtgatagagaacgtatgtcgagtttatccctatcagtgatagagaacgtatgtcgagtttactccctatcagtgatagagaacgtatgtcgaggtaggcgtgtacggtgggaggcctatataagcagagctcgtttagtgaaccgtcagatcgccttcgaatcccggccgggaacggtgcattggaacgcggattccccgtgccaagagtgacgtaagtaccgcctatagagtctataggcccacaaaaaatgctttcttcttttaatatacttttttgtttatcttatttctaatactttccctaatctctttctttcagggcaataatgatacaatgtatcatgcctctttgcaccattctaaagaataacagtgataatttctgggttaaggcaatagcaatatttctgcatataaatatttctgcatataaattgtaactgatgtaagaggtttcatattgctaatagcagctacaatccagctaccattctgcttttattttatggttgggataaggctggattattctgagtccaagctaggcccttttgctaatcatgttcatacctcttatcttcctcccacagctcctgggcaacgtgctggtctgtgtgctggcccatcactttggcaaagaattgggattcgaaatcgattgaattc

SEQ ID NO: 8 - DNA, 887 bp, Artificial sequence
  SpeI-SV40p-optiBSD-SV40pA-PvuII-AgeI
actagtgtgtgtcagttagggtgtggaaagtccccaggctccccagcaggcagaagtatgcaaagcatgcatctcaattagtcagcaaccaggtgtggaaagtccccaggctccccagcaggcagaagtatgcaaagcatgcatctcaattagtcagcaaccatagtcccgcccctaactccgcccatcccgcccctaactccgcccagttccgcccattctccgccccatggctgactaattttttttatttatgcagaggccgaggccgcctctgcctctgagctattccagaagtagtgaggaggcttttttggaggccataggcttttgcaaaaagctatggctaaaccattgtcccaagaggaaagcaccctcattgaaagagcaactgctacaatcaatagtattcctatcagcgaagattattctgtcgcttctgctgctctctctagtgatggtcgtatttttacaggtgtcaatgtatatcattttacaggaggaccatgtgctgaacttgtggtgcttggaactgcggcggcggcggcagcaggcaacctgacttgtatagtcgctatcggaaatgagaacaggggcattttaagtccctgcggaagatgccgacaggtgcttcttgacctccatcctggtatcaaagccatagtgaaagacagtgatggacagccgacggcagttgggattcgtgaattgctgccctctggttatgtgtgggagggctaaaacttgtttattgcagcttataatggttacaaataaagcaatagcatcacaaatttcacaaataaagcatttttttcactgcattctagttgtggtttgtccaaactcatcaatgtatcttacctaggcagctgtccggaaccggt

SEQ ID NO: 9 - DNA, 633 bp, Artificial sequence
  CymR coding sequence
atcgatgccaccatgtctccaaagaggagaacccaggcagagagggcaatggagacacagggcaagctgatcgccgccgccctgggcgtgctgagggagaagggatacgcaggcttccgcatcgccgatgtgccaggagccgccggcgtgtcccggggcgcacagtctcaccacttccctaccaagctggagctgctgctggccacatttgagtggctgtatgagcagatcaccgagaggagccgcgccaggctggcaaagctgaagccagaggacgatgtgatccagcagatgctggacgatgccgccgagttctttctggacgatgactttagcatctccctggatctgatcgtggccgccgatagagaccccgccctgagggagggcatccagaggacagtggagagaaacaggttcgtggtggaggatatgtggctgggcgtgctggtgtctcgcggcctgagccgggatgacgcagaggacatcctgtggctgatctttaacagcgtgcggggcctggccgtgagatccctgtggcagaaggacaaggagcggttcgagcgcgtgcggaattccaccctggagatcgccagagagaggtacgccaagtttaagagatgataactcgag

SEQ ID NO: 10 - DNA, 1496 bp, Artificial sequence
  SpeI-SV40p-optiHygroR-SV40pA-AgeI
actagtgtgtgtcagttagggtgtggaaagtccccaggctccccagcaggcagaagtatgcaaagcatgcatctcaattagtcagcaaccaggtgtggaaagtccccaggctccccagcaggcagaagtatgcaaagcatgcatctcaattagtcagcaaccatagtcccgcccctaactccgcccatcccgcccctaactccgcccagttccgcccattctccgccccatggctgactaattttttttatttatgcagaggccgaggccgcctctgcctctgagctattccagaagtagtgaggaggcttttttggaggccataggcttttgcaaaaagctatgaaaaagcctgaactcacagcgacttctgttgagaagtttctgatcgaaaagttcgacagcgttagcgacctgatgcagctctcggagggcgaggaatctagggctttcagcttcgatgtaggagggcgtggatatgtcctgcgggtaaatagctgcgccgatggtttctacaaagatcgttatgtttatcggcactttgcatcggctgcgctcccgattcccgaagtgcttgacattggggagttcagcgagagcctgacctattgcatctcccgccgcgcacagggcgtaactttgcaagacctccctgaaaccgaactgcccgctgttctacaacctgtcgcggaggctatggacgctattgctgctgccgatctttcccagacttccgggttcggcccatttggaccgcaaggaatcggtcaatacactacatggcgtgatttcatttgcgcgattgctgatccccatgtgtatcattggcaaactgtgatggatgataccgtcagcgcgagtgtcgcgcaggctctcgatgagctgatgctttgggccgaggattgccccgaagttcgccacttggtccacgcggatttcggcagcaacaatgtcctgacagataatggccgcataacagcggtcattgattggagcgaagctatgttcggggattcccaatacgaggtcgctaacatctttttctggcgtccttggttggcttgtatggagcagcaaacgcgctactttgaaagacgacatccagagcttgcaggatcgcctcggctccgggcgtatatgctccgcattggtcttgaccaactctatcagagcttggtggacggcaatttcgatgatgctgcttgggcgcagggtcgatgtgatgcaatcgtccgaagtggagccgggactgtcgggcgaacacaaatcgcccgcagaagcgcagccgtctggaccgatggctgtgtagaagttctcgccgatagtggaaacagacgcccctctactcgtccgagggcaaaggaatagaacttgtttattgcagcttataatggttacaaataaagcaatagcatcacaaatttcacaaataaagcatttttttcactgcattctagttgtggtttgtccaaactcatcaatgtatcttaaccggt

SEQ ID NO: 11 - DNA, 1979 bp, Artificial sequence
  MluI-CAGGS-BGI(C&R)-MCS-SV40pA-AgeI
acgcgtgacattgattattgacatgttattaatagtaatcaattacggggtcattagttcatagcccatatatggagttccgcgttacataacttacggtaaatggcccgcctggctgaccgcccaacgacccccgcccattgacgtcaataatgacgtatgttcccatagtaacgccaatagggactttccattgacgtcaatgggtggagtatttacggtaaactgcccacttggcagtacatcaagtgtatcatatgccaagtacgccccctattgacgtcaatgacggtaaatggcccgcctggcattatgcccagtacatgaccttatgggactttcctacttggcagtacatctacgtattagtcatcgctattaccatggtcgaggtgagccccacgttctgcttcactctccccatctcccccccctccccacccccaattttgtatttatttattttttaattattttgtgcagcgatgggggcggggggggggggggggcgcgcgccaggcggggcggggcggggcgaggggcggggcggggcgaggcggagaggtgcggcggcagccaatcagagcggcgcgctccgaaagtttccttttatggcgaggcggcggcggcggcggccctataaaaagcgaagcgcgcggcgggcgttcgaaggagtcgctgcgacgctgccttcgccccgtgccccgctccgccgccgcctcgcgccgcccgccccggctctgactgaccgcgttactcccacaggtgagcgggcgggacggcccttctcctccgggctgtaattagcgcttggtttaatgacggcttgtttcttttctgtggctgcgtgaaagccttgaggggctccgggagggccctttgtgcggggggagcggctcggggggtgcgtgcgtgtgtgtgtgcgtggggagcgccgcgtgcggctccgcgctgcccggcggctgtgagcgctgcgggcgcggcgcggggctttgtgcgctccgcagtgtgcgcgaggggagcgcggccgggggcggtgccccgcggtgcggggggggctgcgaggggaacaaaggctgcgtgcggggtgtgtgcgtgggggggtgagcagggggtgtgggcgcgtcggtcgggctgcaaccccccctgcacccccctccccgagttgctgagcacggcccggcttcgggtgcggggctccgtacggggcgtggcgcggggctcgccgtgccgggcggggggtggcggcaggtgggggtgccgggcggggcggggccgcctcgggccggggagggctcgggggaggggcgcggcggcccccggagcgccggcggctgtcgaggcgcggcgagccgcagccattgccttttatggtaatcgtgcgagagggcgcagggacttcctttgtcccaaatctgtgcggagccgaaatctgggaggcgccgccgcaccccctctagcgggcgcggggcgaagcggtgcggcgccggcaggaaggaaatgggcggggagggccttcgtgcgtcgccgcgccgccgtccccttctccctctccagcctcggggctgtccgcggggggacggctgccttcgggggggacggggcagggcggggttcggcttctggcgtgtgaccggcggctcttgagcctctgctaaccatgttcatgccttcttctttttcctacagcttcgaacctgggcaacgtgctggttattgtgctgtctcatcattttggcaaaatcgattgaattctggccaagtggatccgctagctctagagtcgacggtaccagtactaagcttgcctcgaggatatcccatggagatctatggggacatcatgaagccccttgagcatctgacttctggctaataaaggaaatttattttcattgcaatagtgtgttggaattttttgtgtctctcactcggaaggacatatgggagcatgccctaggcagctgtccggaaccggt

SEQ ID NO: 12 - DNA, 768 bp, Artificial sequence
  rtTA 3G coding sequence
atcgatgccaccatgagccgcctggataagtccaaagtgatcaactctgccctggagctgctgaatggagtgggaatcgagggactgaccacaaggaagctggcacagaagctgggagtggagcagcctaccctgtactggcacgtgaagaacaagcgcgccctgctggacgcactgccaatcgagatgctggatcggcaccacacacacagctgcccactggagggagagtcctggcaggattttctgcggaacaatgccaagtcttatagatgtgcactgctgagccacagggacggagcaaaggtgcacctgggaaccaggcccacagagaagcagtacgagaccctggagaaccagctggccttcctgtgccagcagggcttttccctggagaatgccctgtatgccctgtctgccgtgggccactttaccctgggatgcgtgctggaggagcaggagcaccaggtggccaaggaggagagagagacaccaaccacagatagcatgccccctctgctgaagcaggccatcgagctgttcgacaggcagggagcagagccagccttcctgtttggcctggagctgatcatctgcggcctggagaagcagctgaagtgtgagtccggaggacctacagacgcactggacgatttcgacctggatatgctgccagccgatgccctggacgattttgacctggatatgctgcccgccgacgccctggatgactttgacctggacatgctgcctggctgataactcgag

SEQ ID NO: 13 - DNA, 765 bp, Artificial sequence
  rtTA adv coding sequence
atcgatgccaccatgtccagactggacaagagcaaagtcataaacggcgctctggaattactcaatggagtcggtatcgaaggcctgacgacaaggaaactcgctcaaaagctgggagttgagcagcctaccctgtactggcacgtgaagaacaagcgggccctgctcgatgccctgccaatcgagatgctggacaggcatcatacccacttctgccccctggaaggcgagtcatggcaagactttctgcggaacaacgccaagtcattccgctgtgctctcctctcacatcgcgacggggctaaagtgcatctcggcacccgcccaacagagaaacagtacgaaaccctggaaaatcagctcgcgttcctgtgtcagcaaggcttctccctggagaacgcactgtacgctctgtccgccgtgggccactttacactgggctgcgtattggaggaacaggagcatcaagtagcaaaagaggaaagagagacacctaccaccgattctatgcccccacttctgagacaagcaattgagctgttcgaccggcagggagccgaacctgccttccttttcggcctggaactaatcatatgtggcctggagaaacagctaaagtgcgaaagcggcgggccggccgacgcccttgacgattttgacttagacatgctcccagccgatgcccttgacgactttgaccttgatatgctgcctgctgacgctcttgacgattttgaccttgacatgctccccgggtaactcgag

SEQ ID NO: 14 - DNA, 1320 bp, Artificial sequence
  XhoI-IRES-ECFP-BglII
ctcgaggcccctctccctcccccccccctaacgttactggccgaagccgcttggaataaggccggtgtgcgtttgtctatatgttattttccaccatattgccgtcttttggcaatgtgagggcccggaaacctggccctgtcttcttgacgagcattcctaggggtctttcccctctcgccaaaggaatgcaaggtctgttgaatgtcgtgaaggaagcagttcctctggaagcttcttgaagacaaacaacgtctgtagcgaccctttgcaggcagcggaaccccccacctggcgacaggtgcctctgcggccaaaagccacgtgtataagatacacctgcaaaggcggcacaaccccagtgccacgttgtgagttggatagttgtggaaagagtcaaatggctctcctcaagcgtattcaacaaggggctgaaggatgcccagaaggtaccccattgtatgggatctgatctggggcctcggtgcacatgctttacatgtgtttagtcgaggttaaaaaaacgtctaggccccccgaaccacggggacgtggttttcctttgaaaaacacgatgataatatggccacaaccatggtgagcaagggcgaggagctgttcaccggggtggtgcccatcctggtcgagctggacggcgacgtaaacggccacaagttcagcgtgtccggcgagggcgagggcgatgccacctacggcaagctgaccctgaagttcatctgcaccaccggcaagctgcccgtgccctggcccaccctcgtgaccaccctgacctggggcgtgcagtgcttcagccgctaccccgaccacatgaagcagcacgacttcttcaagtccgccatgcccgaaggctacgtccaggagcgcaccatcttcttcaaggacgacggcaactacaagacccgcgccgaggtgaagttcgagggcgacaccctggtgaaccgcatcgagctgaagggcatcgacttcaaggaggacggcaacatcctggggcacaagctggagtacaactacatcagccacaacgtctatatcaccgccgacaagcagaagaacggcatcaaggccaacttcaagatccgccacaacatcgaggacggcagcgtgcagctcgccgaccactaccagcagaacacccccatcggcgacggccccgtgctgctgcccgacaaccactacctgagcacccagtccgccctgagcaaagaccccaacgagaagcgcgatcacatggtcctgctggagttcgtgaccgccgccgggatcactctcggcatggacgagctgtacaagtaaagatct

SEQ ID NO: 15 - DNA, 1044 bp, Artificial sequence
  SB transposase coding sequence
ggatccgccaccatgggcaagtccaaggagatctctcaggacctgagaaagaggatcgtggatctgcacaagagcggcagctccctgggagcaatctccaagcgcctggcagtgcctcggtctagcgtgcagaccatcgtgcgcaagtacaagcaccacggcaccacacagccttcttatcggagcggccggagaagggtgctgagcccacgcgacgagcggacactggtgcgcaaggtgcagatcaacccccggaccacagccaaggatctggtgaagatgctggaggagaccggcacaaaggtgtccatctctaccgtgaagagagtgctgtacaggcacaacctgaagggccactccgccagaaagaagcctctgctgcagaataggcacaagaaggcaaggctgaggttcgcaaccgcacacggcgacaaggatcgcacattttggcggaacgtgctgtggtctgacgagaccaagatcgagctgttcggccacaatgatcacagatacgtgtggaggaagaagggcgaggcctgcaagcccaagaataccatccctacagtgaagcacggaggaggctccatcatgctgtggggatgttttgcagcaggaggaacaggcgccctgcacaagatcgacggcatcatggatgccgtgcagtatgtggacatcctgaagcagcacctgaagacctctgtgagaaagctgaagctgggcaggaagtgggtgttccagcacgacaacgatccaaagcacacaagcaaggtggtggccaagtggctgaaggacaataaggtgaaggtgctggagtggcccagccagtcccctgatctgaacccaatcgagaatctgtgggccgagctgaagaagagagtgagggcccggagacccaccaacctgacacagctgcaccagctgtgccaggaggagtgggccaagatccacccaaattactgtggcaagctggtggagggctatcccaagaggctgacccaggtgaagcagtttaagggcaacgccacaaagtattgataactcgag

SEQ ID NO: 16 - DNA, 1806 bp, Artificial sequence
  PB transposase coding sequence
ggatccgccaccatgggcagctccctggacgatgagcacatcctgtccgccctgctgcagtctgacgatgagctggtgggcgaggacagcgattccgaggtgagcgaccacgtgtccgaggacgatgtgcagagcgacacagaggaggccttcatcgatgaggtgcacgaggtgcagccaacctctagcggcagcgagatcctggatgagcagaacgtgatcgagcagcctggctcctctctggcctccaataagatcctgaccctgccacagaggacaatccgcggcaagaacaagcactgctggtctaccagcaagcctacacggagatcccgggtgtctgccctgaaccacgtgcggtcccagagaggcccaaccaggatgtgccgcaatatctacgaccccctgctgtgctttaagctgttctttacagatgagatcatcagcgagatcgtgaagtggaccaacgccgagatctccctgaagaggcgcgagagcatgacctccgccacattcagggacaccaatgaggatgagatctacgccttctttggcatcctggtcatgacagccgtgcggaaggacaaccacatgagcaccgacgatctgtttgatagatccctgtctatggtgtacgtgagcgtgatgagcagggaccgcttcgattttctgatccggtgcctgagaatggacgataagtccatccggcctacactgagagagaatgacgtgttcaccccagtgaggaagatctgggatctgtttatccaccagtgtatccagaactacacaccaggagcacacctgaccatcgacgagcagctgctgggcttccggggcagatgcccttttcgcgtgtacatcccaaataagccctctaagtatggcatcaagatcctgatgatgtgcgatagcggcaccaagtacatgatcaacggcatgccatatctgggcaggggcacccagacaaatggcgtgcccctgggcgagtactatgtgaaggagctgtccaagcctgtgcacggctcttgccgcaacatcacatgtgacaattggttcacctctatccccctggccaagaacctgctgcaggagccttataagctgaccatcgtgggcacagtgaggagcaacaagcgcgagatccccgaggtgctgaagaatagcaggtcccgccctgtgggcacatccatgttctgctttgatggcccactgaccctggtgtcttacaagcccaagcctgccaagatggtgtatctgctgagctcctgtgacgaggatgcctctatcaacgagagcaccggcaagccccagatggtcatgtactataatcagacaaagggcggcgtggacaccctggatcagatgtgcagcgtgatgacctgttcccggaagacaaatagatggcctatggccctgctgtacggcatgatcaacatcgcctgcatcaattctttcatcatctatagccacaacgtgtctagcaagggcgagaaggtgcagagcaggaagaagttcatgcgcaatctgtacatgggcctgacatcctcttttatgcggaagagactggaggcccccaccctgaagaggtatctgcgcgacaacatctccaatatcctgcctaaggaggtgccaggcacctccgacgattctacagaggagccagtgaccaagaagcggacctactgcacatattgtccctccaagatccggagaaaggcctctgccagctgcaagaagtgtaagaaagtgatctgtagagagcacaacatcgacatgtgccagtcttgtttttgataactcgag

SEQ ID NO: 17 - DNA, 1320 bp, Artificial sequence
  XhoI-IRES-EGFP-BglII
ctcgaggcccctctccctcccccccccctaacgttactggccgaagccgcttggaataaggccggtgtgcgtttgtctatatgttattttccaccatattgccgtcttttggcaatgtgagggcccggaaacctggccctgtcttcttgacgagcattcctaggggtctttcccctctcgccaaaggaatgcaaggtctgttgaatgtcgtgaaggaagcagttcctctggaagcttcttgaagacaaacaacgtctgtagcgaccctttgcaggcagcggaaccccccacctggcgacaggtgcctctgcggccaaaagccacgtgtataagatacacctgcaaaggcggcacaaccccagtgccacgttgtgagttggatagttgtggaaagagtcaaatggctctcctcaagcgtattcaacaaggggctgaaggatgcccagaaggtaccccattgtatgggatctgatctggggcctcggtgcacatgctttacatgtgtttagtcgaggttaaaaaaacgtctaggccccccgaaccacggggacgtggttttcctttgaaaaacacgatgataatatggccacaaccatggtgagcaagggcgaggagctgttcaccggggtggtgcccatcctggtcgagctggacggcgacgtaaacggccacaagttcagcgtgtccggcgagggcgagggcgatgccacctacggcaagctgaccctgaagttcatctgcaccaccggcaagctgcccgtgccctggcccaccctcgtgaccaccctgacctacggcgtgcagtgcttcagccgctaccccgaccacatgaagcagcacgacttcttcaagtccgccatgcccgaaggctacgtccaggagcgcaccatcttcttcaaggacgacggcaactacaagacccgcgccgaggtgaagttcgagggcgacaccctggtgaaccgcatcgagctgaagggcatcgacttcaaggaggacggcaacatcctggggcacaagctggagtacaactacaacagccacaacgtctatatcatggccgacaagcagaagaacggcatcaaggtgaacttcaagatccgccacaacatcgaggacggcagcgtgcagctcgccgaccactaccagcagaacacccccatcggcgacggccccgtgctgctgcccgacaaccactacctgagcacccagtccgccctgagcaaagaccccaacgagaagcgcgatcacatggtcctgctggagttcgtgaccgccgccgggatcactctcggcatggacgagctgtacaagtaaagatct

SEQ ID NO: 18 - DNA, 3610 bp, Artificial sequence
  SpeI-RSV-LTR-phi-Gag(334)-RRE-cppt-MCS-WPRE-ppt-LTR-SV40pA-       SV40p-optiPuorR-SV40pA-AgeI
actagttaagtagtcttatgcaatactcttgtagtcttgcaacatggtaacgatgagttagcaacatgccttacaaggagagaaaaagcaccgtgcatgccgattggtggaagtaaggtggtacgatcgtgccttattaggaaggcaacagacgggtctgacatggattggacgaaccactgaattgccgcattgcagagatattgtatttaagtgcctagctcgatacataaacgggtctctctggttagaccagatctgagcctgggagctctctggctaactagggaacccactgcttaagcctcaataaagcttgccttgagtgcttcaagtagtgtgtgcccgtctgttgtgtgactctggtaactagagatccctcagacccttttagtcagtgtggaaaatctctagcagtggcgcccgaacagggacttgaaagcgaaagggaaaccagaggagctctctcgacgcaggactcggcttgctgaagcgcgcacggcaagaggcgaggggcggcgactggtgagtacgccaaaaattttgactagcggaggctagaaggagagagatgggtgcgagagcgtcagtattaagcgggggagaattagatcgcgatgggaaaaaattcggttaaggccagggggaaagaaaaaatataaattaaaacatatagtatgggcaagcagggagctagaacgattcgcagttaatcctggcctgttagaaacatcagaaggctgtagacaaatactgggacagctacaaccatcccttcagacaggatcagaagaacttagatcattatataatacagtagcaaccctctattgtgtgcatcaaaggatagagataaaagacaccaaggaagctttagacaagatagaggaagagcaaaacaaaagaatcgatattaggagtagcacccaccaaggcaaagagaagagtggtgcagagagaaaaaagagcagtgggaataggagctttgttccttgggttcttgggagcagcaggaagcactatgggcgcagcgtcaatgacgctgacggtacaggccagacaattattgtctggtatagtgcagcagcagaacaatttgctgagggctattgaggcgcaacagcatctgttgcaactcacagtctggggcatcaagcagctccaggcaagaatcctggctgtggaaagatacctaaaggatcaacagctcctggggatttggggttgctctggaaaactcatttgcaccactgctgtgccttggaatgctagttggagaattcttcgaacctgcaggatggtaccaaggcctttttaaaagaaaaggggggattggggggtacagtgcaggggaaagaatagtagacataatagcaacagacatacaaactaaagaattacaaaaacaaattacaaaaattcaaaattttgtttaaacttaattaatttaaatacgcgttgcgctagctctagacccgggctcgaggtcgaccgggatccgatatcatatgaatcaacctctggattacaaaatttgtgaaagattgactggtattcttaactatgttgctccttttacgctatgtggatacgctgctttaatgcctttgtatcatgctattgcttcccgtatggctttcattttctcctccttgtataaatcctggttgctgtctctttatgaggagttgtggcccgttgtcaggcaacgtggcgtggtgtgcactgtgtttgctgacgcaacccccactggttggggcattgccaccacctgtcagctcctttccgggactttcgctttccccctccctattgccacggcggaactcatcgccgcctgccttgcccgctgctggacaggggctcggctgttgggcactgacaattccgtggtgttgtcggggaagctgacgtcctttccatggctgctcgcctgtgttgccacctggattctgcgcgggacgtccttctgctacgtcccttcggccctcaatccagcggaccttccttcccgcggcctgctgccggctctgcggcctcttccgcgtcttcgccttcgccctcagacgagtcggatctccctttgggccgcctccccgcctggcggccgcttaagaccaatgacttacaaggcagctgtagatcttagccactttttaaaagaaaaggggggactggaagggctaattcactcccaacgaagacaagatctgctttttgcttgtactgggtctctctggttagaccagatctgagcctgggagctctctggctaactagggaacccactgcttaagcctcaataaagcttgccttgagtgcttcaagtagtgtgtgcccgtctgttgtgtgactctggtaactagagatccctcagacccttttagtcagtgtggaaaatctctagcaggcgatcgcaacttgtttattgcagcttataatggttacaaataaagcaatagcatcacaaatttcacaaataaagcatttttttcactgcattctagttgtggtttgtccaaactcatcaatgtatcttacctagtgtgtgtcagttagggtgtggaaagtccccaggctccccagcaggcagaagtatgcaaagcatgcatctcaattagtcagcaaccaggtgtggaaagtccccaggctccccagcaggcagaagtatgcaaagcatgcatctcaattagtcagcaaccatagtcccgcccctaactccgcccatcccgcccctaactccgcccagttccgcccattctccgccccatggctgactaattttttttatttatgcagaggccgaggccgcctctgcctctgagctattccagaagtagtgaggaggcttttttggaggccataggcttttgcaaaaagctatgactgagtacaagcccacggtgcgcctcgccacccgcgacgatgttcctagagccgtccgcaccctcgccgccgcgttcgccgactaccccgccacgcgccacaccgtagaccctgaccgccacatcgagagggtcacagagctgcaagagctgtttctcacgcgcgtcgggctcgacatcggcaaggtgtgggtcgcggacgacggcgcagcggtggcggtctggaccacgccggagagcgtcgaagcgggggcggtgttcgccgagatcggcccgcgcatggccgagttgagcggttcccggctggccgcgcagcaacagatggagggacttctggcaccgcaccgacccaaggagcccgcgtggttcctggctaccgtcggtgtctcgcccgaccaccagggcaagggtctgggctccgccgtcgttctccccggagtggaggcagccgagagagccggggtgcccgcctttctggaaacctccgcgccccgcaacctccccttctacgagcggctcggcttcaccgtcaccgccgatgtcgaggtgcccgaaggaccgcgtacctggtgcatgacccgcaagcccggtgcctgaaacttgtttattgcagcttataatggttacaaataaagcaatagcatcacaaatttcacaaataaagcatttttttcactgcattctagttgtggtttgtccaaactcatcaatgtatcttaaccggt

SEQ ID NO: 19 - DNA, 301 bp, Artificial sequence
  TRE3G response element sequence
tccctatcagtgatagagaacgtatgaagagtttactccctatcagtgatagagaacgtatgcagactttactccctatcagtgatagagaacgtataaggagtttactccctatcagtgatagagaacgtatgaccagtttactccctatcagtgatagagaacgtatctacagtttactccctatcagtgatagagaacgtatatccagtttactccctatcagtgatagagaacgtattaggcgtgtacggtgggcgcctataaaagcagagctcgtttagtgaaccgtcagatcgcc

SEQ ID NO: 20 - DNA, 344 bp, Artificial sequence
  TRE3G-CuO response element sequence
tccctatcagtgatagagaacgtatgaagagtttactccctatcagtgatagagaacgtatgcagactttactccctatcagtgatagagaacgtataaggagtttactccctatcagtgatagagaacgtatgaccagtttactccctatcagtgatagagaacgtatctacagtttactccctatcagtgatagagaacgtatatccagtttactccctatcagtgatagagaacgtattaggcgtgtacggtgggcgcctataaaagcagagctcgtttagtgaaccgtcagatcgcctggagcaattccacatacaaacagaccagattgtctgtttgtt

SEQ ID NO: 21 - DNA, 307 bp, Artificial sequence
  TREadv response element sequence
tccctatcagtgatagagaacgtatgtcgagtttactccctatcagtgatagagaacgatgtcgagtttactccctatcagtgatagagaacgtatgtcgagtttactccctatcagtgatagagaacgtatgtcgagtttactccctatcagtgatagagaacgtatgtcgagtttatccctatcagtgatagagaacgtatgtcgagtttactccctatcagtgatagagaacgtatgtcgaggtaggcgtgtacggtgggaggcctatataagcagagctcgtttagtgaaccgtcagatcgcc

SEQ ID NO: 22 - DNA, 352 bp, Artificial sequence
  TREadv-CuO response element sequence
tccctatcagtgatagagaacgtatgtcgagtttactccctatcagtgatagagaacgatgtcgagtttactccctatcagtgatagagaacgtatgtcgagtttactccctatcagtgatagagaacgtatgtcgagtttactccctatcagtgatagagaacgtatgtcgagtttatccctatcagtgatagagaacgtatgtcgagtttactccctatcagtgatagagaacgtatgtcgaggtaggcgtgtacggtgggaggcctatataagcaaccggtgtttagtgaaccgtcagatcgcctggagacgccatcataatacaaacagaccagattgtctgtttgtt

SEQ ID NO: 23 - DNA, 231 bp, Artificial sequence
  SB IR/DR sequence
ttagtgtatgtaaacttctgacccactggaattgtgatacagtgaattataagtgaaataatctgtctgtaaacaattgttggaaaaatgacttgtgtcatgcacaaagtagatgtcctaactgacttgccaaaactattgtttgttaacaagaaatttgtggagtagttgaaaaacgagttttaatgactccaacttaagtgtatgtaaacttccgacttcaactgtata

SEQ ID NO: 24 - DNA, 238 bp, Artificial sequence
  PB 3'ITR
ccctagaaagataatcatattgtgacgtacgttaaagataatcatgcgtaaaattgacgcatgtgttttatcggtctgtatatcgaggtttatttattaatttgaatagatattaagttttattatatttacacttacatactaataataaattcaacaaacaatttatttatgtttatttatttattaaaaaaaaacaaaaactcaaaatttcttctataaagtaacaaaactttta

SEQ ID NO: 25 - DNA, 313 bp, Artificial sequence
  PB 5'ITR
catatctataacaagaaaatatatatataataagttatcacgtaagtagaacacgaaataacaatataattatcgtatgagttaaatcttaaaagtcacgtaaaagataatcatgcgtcattttgactcacgcggttgttatagttcaaaatcagtgacacttaccgcattgacaagcacgcctcacgggagctccaagcggcgactgagatgtcctaaatgcacagcgacggattcgcgctatttagaaagagagagcaatatttcaagaatgcatgcgtcaattttacgcagactatctttctagggttaa

SEQ ID NO: 26 - DNA, 488 bp, Artificial sequence
  BGI intron sequence
tcccggccgggaacggtgcattggaacgcggattccccgtgccaagagtgacgtaagtaccgcctatagagtctataggcccacaaaaaatgctttcttcttttaatatacttttttgtttatcttatttctaatactttccctaatctctttctttcagggcaataatgatacaatgtatcatgcctctttgcaccattctaaagaataacagtgataatttctgggttaaggcaatagcaatatttctgcatataaatatttctgcatataaattgtaactgatgtaagaggtttcatattgctaatagcagctacaatccagctaccattctgcttttattttatggttgggataaggctggattattctgagtccaagctaggcccttttgctaatcatgttcatacctcttatcttcctcccacagctcctgggcaacgtgctggtctgtgtgctggcccatcactttggcaaagaattggga

SEQ ID NO: 27 - DNA, 612 bp, Artificial sequence
  CymR encoding nucleic acid sequence
atgtctccaaagaggagaacccaggcagagagggcaatggagacacagggcaagctgatcgccgccgccctgggcgtgctgagggagaagggatacgcaggcttccgcatcgccgatgtgccaggagccgccggcgtgtcccggggcgcacagtctcaccacttccctaccaagctggagctgctgctggccacatttgagtggctgtatgagcagatcaccgagaggagccgcgccaggctggcaaagctgaagccagaggacgatgtgatccagcagatgctggacgatgccgccgagttctttctggacgatgactttagcatctccctggatctgatcgtggccgccgatagagaccccgccctgagggagggcatccagaggacagtggagagaaacaggttcgtggtggaggatatgtggctgggcgtgctggtgtctcgcggcctgagccgggatgacgcagaggacatcctgtggctgatctttaacagcgtgcggggcctggccgtgagatccctgtggcagaaggacaaggagcggttcgagcgcgtgcggaattccaccctggagatcgccagagagaggtacgccaagtttaagagatga

SEQ ID NO: 28 - DNA, 747 bp, Artificial sequence
  rtTA3G encoding nucleic acid sequence
atgagccgcctggataagtccaaagtgatcaactctgccctggagctgctgaatggagtgggaatcgagggactgaccacaaggaagctggcacagaagctgggagtggagcagcctaccctgtactggcacgtgaagaacaagcgcgccctgctggacgcactgccaatcgagatgctggatcggcaccacacacacagctgcccactggagggagagtcctggcaggattttctgcggaacaatgccaagtcttatagatgtgcactgctgagccacagggacggagcaaaggtgcacctgggaaccaggcccacagagaagcagtacgagaccctggagaaccagctggccttcctgtgccagcagggcttttccctggagaatgccctgtatgccctgtctgccgtgggccactttaccctgggatgcgtgctggaggagcaggagcaccaggtggccaaggaggagagagagacaccaaccacagatagcatgccccctctgctgaagcaggccatcgagctgttcgacaggcagggagcagagccagccttcctgtttggcctggagctgatcatctgcggcctggagaagcagctgaagtgtgagtccggaggacctacagacgcactggacgatttcgacctggatatgctgccagccgatgccctggacgattttgacctggatatgctgcccgccgacgccctggatgactttgacctggacatgctgcctggctga

SEQ ID NO: 29 - DNA, 747 bp, Artificial sequence
  rtTAadv encoding nucleic acid sequence
atgtccagactggacaagagcaaagtcataaacggcgctctggaattactcaatggagtcggtatcgaaggcctgacgacaaggaaactcgctcaaaagctgggagttgagcagcctaccctgtactggcacgtgaagaacaagcgggccctgctcgatgccctgccaatcgagatgctggacaggcatcatacccacttctgccccctggaaggcgagtcatggcaagactttctgcggaacaacgccaagtcattccgctgtgctctcctctcacatcgcgacggggctaaagtgcatctcggcacccgcccaacagagaaacagtacgaaaccctggaaaatcagctcgcgttcctgtgtcagcaaggcttctccctggagaacgcactgtacgctctgtccgccgtgggccactttacactgggctgcgtattggaggaacaggagcatcaagtagcaaaagaggaaagagagacacctaccaccgattctatgcccccacttctgagacaagcaattgagctgttcgaccggcagggagccgaacctgccttccttttcggcctggaactaatcatatgtggcctggagaaacagctaaagtgcgaaagcggcgggccggccgacgcccttgacgattttgacttagacatgctcccagccgatgcccttgacgactttgaccttgatatgctgcctgctgacgctcttgacgattttgaccttgacatgctccccgggtaa

SEQ ID NO: 30 - DNA, 1023 bp, Artificial sequence
  SB transposase encoding nucleic acid sequence
atgggcaagtccaaggagatctctcaggacctgagaaagaggatcgtggatctgcacaagagcggcagctccctgggagcaatctccaagcgcctggcagtgcctcggtctagcgtgcagaccatcgtgcgcaagtacaagcaccacggcaccacacagccttcttatcggagcggccggagaagggtgctgagcccacgcgacgagcggacactggtgcgcaaggtgcagatcaacccccggaccacagccaaggatctggtgaagatgctggaggagaccggcacaaaggtgtccatctctaccgtgaagagagtgctgtacaggcacaacctgaagggccactccgccagaaagaagcctctgctgcagaataggcacaagaaggcaaggctgaggttcgcaaccgcacacggcgacaaggatcgcacattttggcggaacgtgctgtggtctgacgagaccaagatcgagctgttcggccacaatgatcacagatacgtgtggaggaagaagggcgaggcctgcaagcccaagaataccatccctacagtgaagcacggaggaggctccatcatgctgtggggatgttttgcagcaggaggaacaggcgccctgcacaagatcgacggcatcatggatgccgtgcagtatgtggacatcctgaagcagcacctgaagacctctgtgagaaagctgaagctgggcaggaagtgggtgttccagcacgacaacgatccaaagcacacaagcaaggtggtggccaagtggctgaaggacaataaggtgaaggtgctggagtggcccagccagtcccctgatctgaacccaatcgagaatctgtgggccgagctgaagaagagagtgagggcccggagacccaccaacctgacacagctgcaccagctgtgccaggaggagtgggccaagatccacccaaattactgtggcaagctggtggagggctatcccaagaggctgacccaggtgaagcagtttaagggcaacgccacaaagtattga

SEQ ID NO: 31 - DNA, 1785 bp, Artificial sequence
  PB transposase encoding nucleic acid sequence
atgggcagctccctggacgatgagcacatcctgtccgccctgctgcagtctgacgatgagctggtgggcgaggacagcgattccgaggtgagcgaccacgtgtccgaggacgatgtgcagagcgacacagaggaggccttcatcgatgaggtgcacgaggtgcagccaacctctagcggcagcgagatcctggatgagcagaacgtgatcgagcagcctggctcctctctggcctccaataagatcctgaccctgccacagaggacaatccgcggcaagaacaagcactgctggtctaccagcaagcctacacggagatcccgggtgtctgccctgaaccacgtgcggtcccagagaggcccaaccaggatgtgccgcaatatctacgaccccctgctgtgctttaagctgttctttacagatgagatcatcagcgagatcgtgaagtggaccaacgccgagatctccctgaagaggcgcgagagcatgacctccgccacattcagggacaccaatgaggatgagatctacgccttctttggcatcctggtcatgacagccgtgcggaaggacaaccacatgagcaccgacgatctgtttgatagatccctgtctatggtgtacgtgagcgtgatgagcagggaccgcttcgattttctgatccggtgcctgagaatggacgataagtccatccggcctacactgagagagaatgacgtgttcaccccagtgaggaagatctgggatctgtttatccaccagtgtatccagaactacacaccaggagcacacctgaccatcgacgagcagctgctgggcttccggggcagatgcccttttcgcgtgtacatcccaaataagccctctaagtatggcatcaagatcctgatgatgtgcgatagcggcaccaagtacatgatcaacggcatgccatatctgggcaggggcacccagacaaatggcgtgcccctgggcgagtactatgtgaaggagctgtccaagcctgtgcacggctcttgccgcaacatcacatgtgacaattggttcacctctatccccctggccaagaacctgctgcaggagccttataagctgaccatcgtgggcacagtgaggagcaacaagcgcgagatccccgaggtgctgaagaatagcaggtcccgccctgtgggcacatccatgttctgctttgatggcccactgaccctggtgtcttacaagcccaagcctgccaagatggtgtatctgctgagctcctgtgacgaggatgcctctatcaacgagagcaccggcaagccccagatggtcatgtactataatcagacaaagggcggcgtggacaccctggatcagatgtgcagcgtgatgacctgttcccggaagacaaatagatggcctatggccctgctgtacggcatgatcaacatcgcctgcatcaattctttcatcatctatagccacaacgtgtctagcaagggcgagaaggtgcagagcaggaagaagttcatgcgcaatctgtacatgggcctgacatcctcttttatgcggaagagactggaggcccccaccctgaagaggtatctgcgcgacaacatctccaatatcctgcctaaggaggtgccaggcacctccgacgattctacagaggagccagtgaccaagaagcggacctactgcacatattgtccctccaagatccggagaaaggcctctgccagctgcaagaagtgtaagaaagtgatctgtagagagcacaacatcgacatgtgccagtcttgtttttga

SEQ ID NO: 32 - DNA, 38 bp, Artificial sequence
  C-VSVG-F
gctcatcgatgccaccatgaagtgccttttgtacttag

SEQ ID NO: 33 - DNA, 35 bp, Artificial sequence
  C-VSVG-R
caggctcgagctattactttccaagtcggttcatc

SEQ ID NO: 34 - DNA, 34 bp, Artificial sequence
  C-rev-F
cgatatcgatgccaccatggcaggaagaagcgga

SEQ ID NO: 35 - DNA, 34 bp, Artificial sequence
  C-rev-R
catgctcgagttactattctttagctcctgactc

SEQ ID NO: 36 - DNA, 29 bp, Artificial sequence
  C-RRE-F
catggatctagaaggagctttgttccttg

SEQ ID NO: 37 - DNA, 33 bp, Artificial sequence
  C-RRE-R
caggctcgagaagcttgtgtaattgttaatttc

SEQ ID NO: 38 - DNA, 33 bp, Artificial sequence
  C-GagPol-F
gcacgaattcgccaccatgggtgcgagagcgtc

SEQ ID NO: 39 - DNA, 36 bp, Artificial sequence
  C-GagPol-R
gcagtctagactattaatcctcatcctgtctacttg

SEQ ID NO: 40 - DNA, 29 bp, Artificial sequence
  hPGK-F
catacgcgtgcttgatatcgaattccacg

SEQ ID NO: 41 - DNA, 24 bp, Artificial sequence
  hPGK-R
cagatgaacttcagggtcagcttg

SEQ ID NO: 42 - DNA, 31 bp, Artificial sequence
  Luc-F
tcaggatccatctgcgatctaagtaagcttg

SEQ ID NO: 43 - DNA, 29 bp, Artificial sequence
  Luc-R
tcaactcgagctagaattacacggcgatc

SEQ ID NO: 44 - DNA, 29 bp, Artificial sequence
  F8V1-F
gtcagatcgatgccaccatgcaaatagag

SEQ ID NO: 45 - DNA, 60 bp, Artificial sequence
  F8V1HA-R
cctgctcgagtcatgcataatcaggcacgtcataggggtagctgccgtagaggtcctgtg

SEQ ID NO: 46 - DNA, 37 bp, Artificial sequence
  FP-BDDF8-F
ccattgaaccaagaagcttctctcaaaacccaccagt

SEQ ID NO: 47 - DNA, 37 bp, Artificial sequence
  FP-BDDF8-R
actggtgggttttgagagaagcttcttggttcaatgg

SEQ ID NO: 48 - DNA, 23 bp, Artificial sequence
  Gag-taqman-F01
ggagctagaacgattcgcagtta

SEQ ID NO: 49 - DNA, 22 bp, Artificial sequence
  Gag-taqman-R01
tgatcctgtctgaagggatggt

SEQ ID NO: 50 - DNA, 17 bp, Artificial sequence
  Gag-Probe-01
tcctggcctgttagaaa

SEQ ID NO: 51 - DNA, 19 bp, Artificial sequence
  Hygro-taqman-F01
tgctccgcattggtcttga

SEQ ID NO: 52 - DNA, 20 bp, Artificial sequence
  Hygro-taqman-R01
cttcggacgattgcatcaca

SEQ ID NO: 53 - DNA, 15 bp, Artificial sequence
  Hygro-Probe-01
atgctgcttgggcgc

SEQ ID NO: 54 - DNA, 26 bp, Artificial sequence
  REV-taqman-F01
aggaatagaagaagaaggtggagaga

SEQ ID NO: 55 - DNA, 18 bp, Artificial sequence
  REV-taqman-R01
gcacaggctccgcagatc

SEQ ID NO: 56 - DNA, 20 bp, Artificial sequence
  REV-Probe-01
attcgattagtgaacggatc

SEQ ID NO: 57 - DNA, 20 bp, Artificial sequence
  VSVG-taqman-F01
attgcccgtcaagctcagat

SEQ ID NO: 58 - DNA, 22 bp, Artificial sequence
  VSVG-taqman-R01
ccgtctgcttgaatagccttgt

SEQ ID NO: 59 - DNA, 22 bp, Artificial sequence
  VSVG-Probe-01
tacaagtcaaaatgcccaagag